European Patent Application EP 4 226 945 A1, published August 16, 2023. Title: A pharmaceutical combination for treating tumor. Applicant: Chiome Bioscience Inc. The sequence listing filed with the application follows.

SEQUENCE LISTING (46 sequences)

SEQ ID NO: 1 - DNA, 1532 bp, Homo sapiens
  CDS (154)..(1305)
gagagcgcagcgcgcagcccggtgcagccctggctttcccctcgctgcgcgcccgcgccccctttcgcgtccgcaaccagaagcccagtgcggcgccaggagccggacccgcgcccgcaccgctcccgggaccgcgaccccggccgcccagagatgaccgcgaccgaagccctcctgcgcgtcctcttgctcctgctggctttcggccacagcacctatggggctgaatgcttcccggcctgcaacccccaaaatggattctgcgaggatgacaatgtttgcaggtgccagcctggctggcagggtcccctttgtgaccagtgcgtgacctctcccggctgccttcacggactctgtggagaacccgggcagtgcatttgcaccgacggctgggacggggagctctgtgatagagatgttcgggcctgctcctcggccccctgtgccaacaacaggacctgcgtgagcctggacgatggcctctatgaatgctcctgtgcccccgggtactcgggaaaggactgccagaaaaaggacgggccctgtgtgatcaacggctccccctgccagcacggaggcacctgcgtggatgatgagggccgggcctcccatgcctcctgcctgtgcccccctggcttctcaggcaatttctgcgagatcgtggccaacagctgcacccccaacccatgcgagaacgacggcgtctgcactgacattgggggcgacttccgctgccggtgcccagccggcttcatcgacaagacctgcagccgcccggtgaccaactgcgccagcagcccgtgccagaacgggggcacctgcctgcagcacacccaggtgagctacgagtgtctgtgcaagcccgagttcacaggtctcacctgtgtcaagaagcgcgcgctgagcccccagcaggtcacccgtctgcccagcggctatgggctggcctaccgcctgacccctggggtgcacgagctgccggtgcagcagccggagcaccgcatcctgaaggtgtccatgaaagagctcaacaagaaaacccctctcctcaccgagggccaggccatctgcttcaccatcctgggcgtgctcaccagcctggtggtgctgggcactgtgggtatcgtcttcctcaacaagtgcgagacctgggtgtccaacctgcgctacaaccacatgctgcggaagaagaagaacctgctgcttcagtacaacagcggggaggacctggccgtcaacatcatcttccccgagaagatcgacatgaccaccttcagcaaggaggccggcgacgaggagatctaagcagcgttcccacagccccctctagattcttggagttccgcagagcttactatacgcggtctgtcctaatctttgtggtgttcgctatctcttgtgtcaaatctggtgaacgctacgcttacatatattgtctttgtgctgctgtgtgacaaacgcaatgcaaaaacaatcctctttctctctcttaatgcatgatacagaataataataagaatttcatctttaaa

SEQ ID NO: 2 - protein, 383 aa, Homo sapiens
MTATEALLRVLLLLLAFGHSTYGAECFPACNPQNGFCEDDNVCRCQPGWQGPLCDQCVTSPGCLHGLCGEPGQCICTDGWDGELCDRDVRACSSAPCANNRTCVSLDDGLYECSCAPGYSGKDCQKKDGPCVINGSPCQHGGTCVDDEGRASHASCLCPPGFSGNFCEIVANSCTPNPCENDGVCTDIGGDFRCRCPAGFIDKTCSRPVTNCASSPCQNGGTCLQHTQVSYECLCKPEFTGLTCVKKRALSPQQVTRLPSGYGLAYRLTPGVHELPVQQPEHRILKVSMKELNKKTPLLTEGQAICFTILGVLTSLVVLGTVGIVFLNKCETWVSNLRYNHMLRKKKNLLLQYNSGEDLAVNIIFPEKIDMTTFSKEAGDEEI

SEQ ID NO: 3 - protein, 5 aa, Mus musculus
DTYIH

SEQ ID NO: 4 - protein, 17 aa, Mus musculus
RIDPPNGNLKYDPKFQG

SEQ ID NO: 5 - protein, 8 aa, Mus musculus
SDGYSFAY

SEQ ID NO: 6 - protein, 16 aa, Mus musculus
RSSKSLLHSNGNTYLY

SEQ ID NO: 7 - protein, 7 aa, Mus musculus
RMSNLAS

SEQ ID NO: 8 - protein, 9 aa, Mus musculus
MQHVEYPFT

SEQ ID NO: 9 - protein, 5 aa, Mus musculus
DYAMH

SEQ ID NO: 10 - protein, 17 aa, Mus musculus
VISTYYGNTNYNQKFKG

SEQ ID NO: 11 - protein, 12 aa, Mus musculus
GGLREYYYAMDY

SEQ ID NO: 12 - protein, 17 aa, Mus musculus
KSSQSLLNSSNQKNYLA

SEQ ID NO: 13 - protein, 7 aa, Mus musculus
FASTRES

SEQ ID NO: 14 - protein, 9 aa, Mus musculus
QQHYSTPPT

SEQ ID NO: 15 - DNA, 354 bp, Mus musculus
  CDS (1)..(354)
gaggttcagctgcagcagtctggggcagagcttgtgaagccaggggcctcagtcaagttgtcctgcacagcttctggcttcaacattagagacacctatatacactgggtgaagcagaggcctgagcagggcctggagtggattggaaggattgatcctccgaatggtaatcttaaatatgacccgaagttccagggcaaggccactataacagcagacacatcctccaacacagcctacctgcagttcagcagcctgacatctgaggacactgccgtctattactgtgcaaggtctgatggttactcctttgcttactggggccaagggactctggtcactgtctctgcagcc

SEQ ID NO: 16 - protein, 118 aa, Mus musculus
EVQLQQSGAELVKPGASVKLSCTASGFNIRDTYIHWVKQRPEQGLEWIGRIDPPNGNLKYDPKFQGKATITADTSSNTAYLQFSSLTSEDTAVYYCARSDGYSFAYWGQGTLVTVSAA

SEQ ID NO: 17 - DNA, 336 bp, Mus musculus
  CDS (1)..(336)
gatattgtgatgactcaggctgcaccctctgtacctgtcactcctggagagtcagtatccatctcctgcaggtctagtaagagtctcctgcatagtaatggcaacacttacttgtattggttcctgcagaggccaggccagtctcctcagctcctgatatatcggatgtccaaccttgcctcaggagtcccagacaggttcagtggcagtgggtcaggaactgctttcacactgagaatcagtagagtggaggctgaggatgtgggtgtttattactgtatgcaacatgtagaatatccattcacgttcggctcggggacaaagttggaaataaaa

SEQ ID NO: 18 - protein, 112 aa, Mus musculus
DIVMTQAAPSVPVTPGESVSISCRSSKSLLHSNGNTYLYWFLQRPGQSPQLLIYRMSNLASGVPDRFSGSGSGTAFTLRISRVEAEDVGVYYCMQHVEYPFTFGSGTKLEIK

SEQ ID NO: 19 - DNA, 363 bp, Mus musculus
  CDS (1)..(363)
caggtccagctgcagcagtctgggcctgagctggtgaggcctggggtctcagtgaagatttcctgcaagggttccggctacacattcactgattatgctatgcactgggtgaagcagagtcatgcaaagagtctagagtggattggagttattagtacttactatggtaatacaaactacaaccagaagtttaagggcaaggccacaatgactgtagacaaatcctccagcacagcctatatggaacttgccagattgacatctgaggattctgccatctattactgtgcaagaggaggattacgagagtattactatgctatggactactggggtcaaggaacctcagtcaccgtctcctca

SEQ ID NO: 20 - protein, 121 aa, Mus musculus
QVQLQQSGPELVRPGVSVKISCKGSGYTFTDYAMHWVKQSHAKSLEWIGVISTYYGNTNYNQKFKGKATMTVDKSSSTAYMELARLTSEDSAIYYCARGGLREYYYAMDYWGQGTSVTVSS

SEQ ID NO: 21 - DNA, 339 bp, Mus musculus
  CDS (1)..(339)
gacattgtgatgacacagtctccatcctccctggctatgtcagtaggacagaaggtcactatgagctgcaagtccagtcagagccttttaaatagtagcaatcaaaagaactatttggcctggtaccagcagaaaccaggacagtctcctaaacttctggtatactttgcatccactagggaatctggggtccctgatcgcttcataggcagtggatctgggacagatttcactcttaccatcagcagtgtgcaggctgaagacctggcagattacttctgtcagcaacattatagcactcctcccacgttcggtgctgggaccaagctggagctgaaa

SEQ ID NO: 22 - protein, 113 aa, Mus musculus
DIVMTQSPSSLAMSVGQKVTMSCKSSQSLLNSSNQKNYLAWYQQKPGQSPKLLVYFASTRESGVPDRFIGSGSGTDFTLTISSVQAEDLADYFCQQHYSTPPTFGAGTKLELK

SEQ ID NO: 23 - DNA, 351 bp, Artificial
  Recombinant DNA
  CDS (1)..(351)
caggttcagctggtgcagtctggggcagaggtgaagaagccagggtcctcagtcaaggtctcctgcaaggcttctggcttcaacattagagacacctatatacactgggtgcggcaggcccctggacagggcctggagtggattggaaggattgatcctccgaatggtaatcttaaatatgacccgaagttccagggcaaggccactataacagcagacacatccacgagcacagcctacatggagttcagcagcctgagatctgaggacactgccgtctattactgtgcaaggtctgatggttactcctttgcttactggggccaagggactctggtcactgtctcttca

SEQ ID NO: 24 - protein, 117 aa, Artificial
  Synthetic Construct (Recombinant Protein)
QVQLVQSGAEVKKPGSSVKVSCKASGFNIRDTYIHWVRQAPGQGLEWIGRIDPPNGNLKYDPKFQGKATITADTSTSTAYMEFSSLRSEDTAVYYCARSDGYSFAYWGQGTLVTVSS

SEQ ID NO: 25 - DNA, 351 bp, Artificial
  Recombinant DNA
  CDS (1)..(351)
caggttcagctggtgcagtctggggcagaggtgaagaagccagggtcctcagtcaaggtctcctgcaaggcttctggcttcaacattagagacacctatatacactgggtgcggcaggcccctggacagggcctggagtggattggaaggattgatcctccgaatggtaatcttaaatatgacccgaagttccagggcaaggccactataacagcagacacatccacgagcacagcctacatggagctgagcagcctgagatctgaggacactgccgtctattactgtgcaaggtctgatggttactcctttgcttactggggccaaggaactctggtcactgtctcttca

SEQ ID NO: 26 - protein, 117 aa, Artificial
  Synthetic Construct (Recombinant Protein)
QVQLVQSGAEVKKPGSSVKVSCKASGFNIRDTYIHWVRQAPGQGLEWIGRIDPPNGNLKYDPKFQGKATITADTSTSTAYMELSSLRSEDTAVYYCARSDGYSFAYWGQGTLVTVSS

SEQ ID NO: 27 - DNA, 336 bp, Artificial
  Recombinant DNA
  CDS (1)..(336)
gatattgtgatgactcagtctccactctctctgcctgtcactcctggagagccggcctccatctcctgcaggtctagcaagagtctcctgcatagtaatggcaacacttacttgtattggttcctgcagaagccaggccagtctcctcagctcctgatatatcggatgtccaaccttgcctcaggagtcccagacaggttcagtggcagtgggtcaggaactgctttcacactgaaaatcagtagagtggaggctgaggatgtgggtgtttattactgtatgcaacatgtagaatatccattcacgttcggccaagggacaaaggtggaaatcaaa

SEQ ID NO: 28 - protein, 112 aa, Artificial
  Synthetic Construct (Recombinant Protein)
DIVMTQSPLSLPVTPGEPASISCRSSKSLLHSNGNTYLYWFLQKPGQSPQLLIYRMSNLASGVPDRFSGSGSGTAFTLKISRVEAEDVGVYYCMQHVEYPFTFGQGTKVEIK

SEQ ID NO: 29 - DNA, 363 bp, Artificial
  Recombinant DNA
  CDS (1)..(363)
caagtccagctggtgcagtctggggctgaagtgaagaagcctggggcctcagtgaaagtctcctgcaaggcttccggctacacattcactgattatgctatgcactgggtgcgacaggcccctggacaaggcctggagtggattggagttattagtacttactatggtaatacaaactacaaccagaagtttaagggcaaggccacaatgactgtcgacacatccaccagcacagcctatatggaacttaggagcttgagatctgacgatactgccgtgtattactgtgcaagaggaggattgcgagagtattactatgctatggactactggggtcaaggaaccatggtcaccgtctcctca

SEQ ID NO: 30 - protein, 121 aa, Artificial
  Synthetic Construct (Recombinant Protein)
QVQLVQSGAEVKKPGASVKVSCKASGYTFTDYAMHWVRQAPGQGLEWIGVISTYYGNTNYNQKFKGKATMTVDTSTSTAYMELRSLRSDDTAVYYCARGGLREYYYAMDYWGQGTMVTVSS

SEQ ID NO: 31 - DNA, 363 bp, Artificial
  Recombinant DNA
  CDS (1)..(363)
caagtccagctggtgcagtctggggctgaagtgaagaagcctggggcctcagtgaaagtctcctgcaagggttccggctacacattcactgattatgctatgcactgggtgcgacaggcccctggacaaggcctggagtggattggagttattagtacttactatggtaatacaaactacaaccagaagtttaagggcaaggccacaatgactgtcgacacatccaccagcacagcctatatggaacttaggagcttgagatctgacgatactgccgtgtattactgtgcaagaggaggattgcgagagtattactatgctatggactactggggtcaaggaaccatggtcaccgtctcctca

SEQ ID NO: 32 - protein, 121 aa, Artificial
  Synthetic Construct (Recombinant Protein)
QVQLVQSGAEVKKPGASVKVSCKGSGYTFTDYAMHWVRQAPGQGLEWIGVISTYYGNTNYNQKFKGKATMTVDTSTSTAYMELRSLRSDDTAVYYCARGGLREYYYAMDYWGQGTMVTVSS

SEQ ID NO: 33 - DNA, 363 bp, Artificial
  Recombinant DNA
  CDS (1)..(363)
caagtccagctggtgcagtctggggctgaagtgaagaagcctggggcctcagtgaaagtctcctgcaaggcttccggctacacattcactgattatgctatgcactgggtgcgacaggcccctggacaaggcctggagtggattggagttattagtacttactatggtaatacaaactacaaccagaagtttaagggcaaggccacaatgactgtcgacaaatccaccagcacagcctatatggaacttaggagcttgagatctgacgatactgccgtgtattactgtgcaagaggaggattgcgagagtattactatgctatggactactggggtcaaggaaccatggtcaccgtctcctca

SEQ ID NO: 34 - protein, 121 aa, Artificial
  Synthetic Construct (Recombinant Protein)
QVQLVQSGAEVKKPGASVKVSCKASGYTFTDYAMHWVRQAPGQGLEWIGVISTYYGNTNYNQKFKGKATMTVDKSTSTAYMELRSLRSDDTAVYYCARGGLREYYYAMDYWGQGTMVTVSS

SEQ ID NO: 35 - DNA, 363 bp, Artificial
  Recombinant DNA
  CDS (1)..(363)
caagtccagctggtgcagtctggggctgaagtgaagaagcctggggcctcagtgaaagtctcctgcaagggttccggctacacattcactgattatgctatgcactgggtgcgacaggcccctggacaaggcctggagtggattggagttattagtacttactatggtaatacaaactacaaccagaagtttaagggcaaggccacaatgactgtcgacaaatccaccagcacagcctatatggaacttaggagcttgagatctgacgatactgccgtgtattactgtgcaagaggaggattgcgagagtattactatgctatggactactggggtcaaggaaccatggtcaccgtctcctca

SEQ ID NO: 36 - protein, 121 aa, Artificial
  Synthetic Construct (Recombinant Protein)
QVQLVQSGAEVKKPGASVKVSCKGSGYTFTDYAMHWVRQAPGQGLEWIGVISTYYGNTNYNQKFKGKATMTVDKSTSTAYMELRSLRSDDTAVYYCARGGLREYYYAMDYWGQGTMVTVSS

SEQ ID NO: 37 - DNA, 363 bp, Artificial
  Recombinant DNA
  CDS (1)..(363)
caagtccagctggtgcagtctggggctgaagtgaagaagcctggggcctcagtgaaagtctcctgcaaggcttccggctacacattcactgattatgctatgcactgggtgcgacaggcccctggacaaggcctggagtggattggagttattagtacttactatggtaatacaaactacaaccagaagtttaagggccgagccacaatgactgtcgacacatccaccagcacagcctatatggaacttaggagcttgagatctgacgatactgccgtgtattactgtgcaagaggaggattgcgagagtattactatgctatggactactggggtcaaggaaccatggtcaccgtctcctca

SEQ ID NO: 38 - protein, 121 aa, Artificial
  Synthetic Construct (Recombinant Protein)
QVQLVQSGAEVKKPGASVKVSCKASGYTFTDYAMHWVRQAPGQGLEWIGVISTYYGNTNYNQKFKGRATMTVDTSTSTAYMELRSLRSDDTAVYYCARGGLREYYYAMDYWGQGTMVTVSS

SEQ ID NO: 39 - DNA, 363 bp, Artificial
  Recombinant DNA
  CDS (1)..(363)
caagtccagctggtgcagtctggggctgaagtgaagaagcctggggcctcagtgaaagtctcctgcaagggttccggctacacattcactgattatgctatgcactgggtgcgacaggcccctggacaaggcctggagtggattggagttattagtacttactatggtaatacaaactacaaccagaagtttaagggccgagccacaatgactgtcgacacatccaccagcacagcctatatggaacttaggagcttgagatctgacgatactgccgtgtattactgtgcaagaggaggattgcgagagtattactatgctatggactactggggtcaaggaaccatggtcaccgtctcctca

SEQ ID NO: 40 - protein, 121 aa, Artificial
  Synthetic Construct (Recombinant Protein)
QVQLVQSGAEVKKPGASVKVSCKGSGYTFTDYAMHWVRQAPGQGLEWIGVISTYYGNTNYNQKFKGRATMTVDTSTSTAYMELRSLRSDDTAVYYCARGGLREYYYAMDYWGQGTMVTVSS

SEQ ID NO: 41 - DNA, 363 bp, Artificial
  Recombinant DNA
  CDS (1)..(363)
caagtccagctggtgcagtctggggctgaagtgaagaagcctggggcctcagtgaaagtctcctgcaaggcttccggctacacattcactgattatgctatgcactgggtgcgacaggcccctggacaaggcctggagtggattggagttattagtacttactatggtaatacaaactacaaccagaagtttaagggccgagccacaatgactgtcgacaaatccaccagcacagcctatatggaacttaggagcttgagatctgacgatactgccgtgtattactgtgcaagaggaggattgcgagagtattactatgctatggactactggggtcaaggaaccatggtcaccgtctcctca

SEQ ID NO: 42 - protein, 121 aa, Artificial
  Synthetic Construct (Recombinant Protein)
QVQLVQSGAEVKKPGASVKVSCKASGYTFTDYAMHWVRQAPGQGLEWIGVISTYYGNTNYNQKFKGRATMTVDKSTSTAYMELRSLRSDDTAVYYCARGGLREYYYAMDYWGQGTMVTVSS

SEQ ID NO: 43 - DNA, 363 bp, Artificial
  Recombinant DNA
  CDS (1)..(363)
caagtccagctggtgcagtctggggctgaagtgaagaagcctggggcctcagtgaaagtctcctgcaagggttccggctacacattcactgattatgctatgcactgggtgcgacaggcccctggacaaggcctggagtggattggagttattagtacttactatggtaatacaaactacaaccagaagtttaagggccgagccacaatgactgtcgacaaatccaccagcacagcctatatggaacttaggagcttgagatctgacgatactgccgtgtattactgtgcaagaggaggattgcgagagtattactatgctatggactactggggtcaaggaaccatggtcaccgtctcctca

SEQ ID NO: 44 - protein, 121 aa, Artificial
  Synthetic Construct (Recombinant Protein)
QVQLVQSGAEVKKPGASVKVSCKGSGYTFTDYAMHWVRQAPGQGLEWIGVISTYYGNTNYNQKFKGRATMTVDKSTSTAYMELRSLRSDDTAVYYCARGGLREYYYAMDYWGQGTMVTVSS

SEQ ID NO: 45 - DNA, 339 bp, Artificial
  Recombinant DNA
  CDS (1)..(339)
gacattgtcatgacacagtctccagactccctggctgtgtcactgggagagagggccactatcaactgcaagtccagtcagagccttctgaatagtagcaatcaaaagaactatttggcctggtaccagcagaaaccaggacagcctcctaaacttctggtctactttgcatccactagggaatctggggtccctgatcgcttcagtggcagtggatctgggacagatttcactcttaccatcagcagtctgcaggctgaagatgtggcagtttactactgtcagcaacattatagcactcctcccacattcggtcaggggaccaagctggagatcaaa

SEQ ID NO: 46 - protein, 113 aa, Artificial
  Synthetic Construct (Recombinant Protein)
DIVMTQSPDSLAVSLGERATINCKSSQSLLNSSNQKNYLAWYQQKPGQPPKLLVYFASTRESGVPDRFSGSGSGTDFTLTISSLQAEDVAVYYCQQHYSTPPTFGQGTKLEIK